European Patent Application EP 4 357 369 A1, published April 24, 2024. Title: PREPARATION AND APPLICATION OF CHIMERIC ANTIGEN RECEPTOR IMMUNE CELL CONSTRUCTED ON BASIS OF GRANZYME B. Applicant: WEST CHINA HOSPITAL, SICHUAN UNIVERSITY. The sequence listing filed with the application follows.

SEQUENCE LISTING (8 sequences)

SEQ ID NO: 1 - protein, 247 aa, Homo sapiens
MQPILLLLAFLLLPRADAGEIIGGHEAKPHSRPYMAYLMIWDQKSLKRCGGFLIRDDFVLTAAHCWGSSINVTLGAHNIKEQEPTQQFIPVKRPIPHPAYNPKNFSNDIMLLQLERKAKRTRAVQPLRLPSNKAQVKPGQTCSVAGWGQTAPLGKHSHTLQEVKMTVQEDRKCESDLRHYYDSTIELCVGDPEIKKTSFKGDSGGPLVCNKVAQGIVSYGRNNGMPPRACTKVSSFVHWIKKTMKRY

SEQ ID NO: 2 - protein, 233 aa, Artificial sequence
  mKate2 red fluorescent protein
MSELIKENMHMKLYMEGTVNNHHFKCTSEGEGKPYEGTQTMRIKAVEGGPLPFAFDILATSFMYGSKTFINHTQGIPDFFKQSFPEGFTWERVTTYEDGGVLTATQDTSLQDGCLIYNVKIRGVNFPSNGPVMQKKTLGWEASTETLYPADGGLEGRADMALKLVGGGHLICNLKTTYRSKKPAKNLKMPGVYYVDRRLERIKEADKETYVEQHEVAVARYCDLPSKLGHKLN

SEQ ID NO: 3 - protein, 22 aa, Artificial sequence
  signal peptide
MAAATGPSFWLGNETLKVPLAL

SEQ ID NO: 4 - protein, 45 aa, Artificial sequence
  CD8 hinge
TTTPAPRPPTPAPTIASQPLSLRPEACRPAAGGAVHTRGLDFACD

SEQ ID NO: 5 - protein, 24 aa, Artificial sequence
  CD28 transmembrane region
IYIWAPLAGTCGVLLLSLVITLYC

SEQ ID NO: 6 - protein, 43 aa, Artificial sequence
  costimulatory molecule derived from 4-1BB
KRGRKKLLYIFKQPFMRPVQTTQEEDGCSCRFPEEEEGGCELR

SEQ ID NO: 7 - protein, 111 aa, Artificial sequence
  cytoplasmic signaling sequence derived from CD3zeta
VKFSRSADAPAYKQGQNQLYNELNLGRREEYDVLDKRRGRDPEMGGKPRRKNPQEGLYNELQKDKMAEAYSEIGMKGERRRGKGHDGLYQGLSTATKDTYDALHMQALPPR

SEQ ID NO: 8 - protein, 474 aa, Artificial sequence
  full length of CAR
MALPVTALLLPLALLLHAARPIIGGHEAKPHSRPYMAYLMIWDQKSLKRCGGFLIRDDFVLTAAHCWGSSINVTLGAHNIKEQEPTQQFIPVKRPIPHPAYNPKNFSNDIMLLQLERKAKRTRAVQPLRLPSNKAQVKPGQTCSVAGWGQTAPLGKHSHTLQEVKMTVQEDRKCESDLRHYYDSTIELCVGDPEIKKTSFKGDSGGPLVCNKVAQGIVSYGRNNGMPPRACTKVSSFVHWIKKTMKRYTTTPAPRPPTPAPTIASQPLSLRPEACRPAAGGAVHTRGLDFACDIYIWAPLAGTCGVLLLSLVITLYCKRGRKKLLYIFKQPFMRPVQTTQEEDGCSCRFPEEEEGGCELRVKFSRSADAPAYKQGQNQLYNELNLGRREEYDVLDKRRGRDPEMGGKPRRKNPQEGLYNELQKDKMAEAYSEIGMKGERRRGKGHDGLYQGLSTATKDTYDALHMQALPPRGSG